European Patent Specification EP 3 227 330 B1, published January 17, 2024. Title: TDP-43 binding polypeptides useful for the treatment of neurodegenerative diseases. Applicant: Université Laval. Application PCT application. The sequence listing filed with the application follows.

SEQUENCE LISTING (53 sequences)

SEQ ID NO: 1 - protein, 118 aa, Artificial Sequence
  E6_VH1 heavy chain variable region
LQESGGGLVQPGGSMKLSCVASGFTSSNYWLNWVRQSPERGLEWVAEIRLKSNNYATNYAESVKGRFTISRDDSKSSVYLQVNNLRAEDTGIYYCTRSTARATPYYFDYWGQGTTVTV

SEQ ID NO: 2 - protein, 118 aa, Artificial Sequence
  E6_VH7 heavy chain variable region
LQQSGGGLVQPGGSMKLSCVASGFTSSNYWLNWVRQSPERGLEWVAEIRLKSNNYATNYAESVKGRFTISRDDSKSSVYLQVNNLRAEDTGIYYCTRSTARATPYYFDYWGQGTTVTV

SEQ ID NO: 3 - protein, 108 aa, Artificial Sequence
  E6_Vk9 light chain variable region
ELTQSPSSLAVSAGEKVTMSCKSSQSLLNSRARKNFLTWYQQKPGQSPKLLIYWASTRESGVPDRFTGSGSGTDFTLTISSVQAEDLAVYYCKQSYNLYTFGGGTKLE

SEQ ID NO: 4 - protein, 97 aa, Artificial Sequence
  C10_VH3 heavy chain variable region
LQESGGGLVQPGGSRKLSCAASGFTFSSFGMHWVRQAPEKGLEWVAYISSGSSTLHYADTVKGRFTISRDNPKNTLFLQMKLPSLCYGLLGPRDHGH

SEQ ID NO: 5 - protein, 97 aa, Artificial Sequence
  C10_VH4 heavy chain variable region
LQQSGGGLVQPGGSRKLSCAASGFTFSSFGMHWVRQAPEKGLEWVAYISSGSSTLHYADTVKGRFTISRDNPKNTLFLQMKLPSLCYGLLGPRDHGH

SEQ ID NO: 6 - protein, 105 aa, Artificial Sequence
  C10_Vk3 light chain variable region
ELTQSPASLAVSLGQRATISYRASKSVSTSGYSYMHWNQQKPGQPPRLLIYLVSNLESGVPARFSGSGSGTDFTLNIHPVEEEDAATYYCQHIRELTRSEGAPSS

SEQ ID NO: 7 - protein, 8 aa, Artificial Sequence
  E6_VH1 CDR1
SSNYWLNW

SEQ ID NO: 8 - protein, 15 aa, Artificial Sequence
  E6_VH1 CDR2
EIRLKSNNYATNYAE

SEQ ID NO: 9 - protein, 9 aa, Artificial Sequence
  E6_VH1 CDR3
RATPYYFDY

SEQ ID NO: 10 - protein, 8 aa, Artificial Sequence
  E6_VH7 CDR1
SSNYWLNW

SEQ ID NO: 11 - protein, 15 aa, Artificial Sequence
  E6_VH7 CDR2
EIRLKSNNYATNYAE

SEQ ID NO: 12 - protein, 9 aa, Artificial Sequence
  E6_VH7 CDR3
RATPYYFDY

SEQ ID NO: 13 - protein, 17 aa, Artificial Sequence
  E6_Vk9 CDR1
KSSQSLLNSRARKNFLT

SEQ ID NO: 14 - protein, 8 aa, Artificial Sequence
  E6_Vk9 CDR2
YWASTRES

SEQ ID NO: 15 - protein, 8 aa, Artificial Sequence
  E6_Vk9 CDR3
KQSYNLYT

SEQ ID NO: 16 - protein, 7 aa, Artificial Sequence
  C10_VH3 CDR1
SSFGMHW

SEQ ID NO: 17 - protein, 13 aa, Artificial Sequence
  C10_VH3 CDR2
YISSGSSTLHYAD

SEQ ID NO: 18 - protein, 9 aa, Artificial Sequence
  C10_VH3 CDR3
FLQMKLPSL

SEQ ID NO: 19 - protein, 7 aa, Artificial Sequence
  C10_VH4 CDR1
SSFGMHW

SEQ ID NO: 20 - protein, 13 aa, Artificial Sequence
  C10_VH4 CDR2
YISSGSSTLHYAD

SEQ ID NO: 21 - protein, 9 aa, Artificial Sequence
  C10_VH4 CDR3
FLQMKLPSL

SEQ ID NO: 22 - protein, 15 aa, Artificial Sequence
  C10_Vk3 CDR1
RASKSVSTSGYSYMH

SEQ ID NO: 23 - protein, 8 aa, Artificial Sequence
  C10_Vk3 CDR2
YLVSNLES

SEQ ID NO: 24 - protein, 8 aa, Artificial Sequence
  C10_Vk3 CDR3
QHIRELTR

SEQ ID NO: 25 - protein, 276 aa, Artificial Sequence
  E6_VH1 Vk9 complete with IGk secretory signal and c-myc peptide
MGDNDIHFAFLSTGVHSQVQLQESGGGLVQPGGSMKLSCVASGFTSSNYWLNWVRQSPERGLEWVAEIRLKSNNYATNYAESVKGRFTISRDDSKSSVYLQVNNLRAEDTGIYYCTRSTARATPYYFDYWGQGTTVTVSSGGGGSGGGGSGGGGSDIELTQSPSSLAVSAGEKVTMSCKSSQSLLNSRARKNFLTWYQQKPGQSPKLLIYWASTRESGVPDRFTGSGSGTDFTLTISSVQAEDLAVYYCKQSYNLYTFGGGTKLEEQKLISEEDLN

SEQ ID NO: 26 - protein, 245 aa, Artificial Sequence
  E6_VH1 Vk9 full
LQESGGGLVQPGGSMKLSCVASGFTSSNYWLNWVRQSPERGLEWVAEIRLKSNNYATNYAESVKGRFTISRDDSKSSVYLQVNNLRAEDTGIYYCTRSTARATPYYFDYWGQGTTVTVSSGGGGSGGGGSGGGGSDIELTQSPSSLAVSAGEKVTMSCKSSQSLLNSRARKNFLTWYQQKPGQSPKLLIYWASTRESGVPDRFTGSGSGTDFTLTISSVQAEDLAVYYCKQSYNLYTFGGGTKLE

SEQ ID NO: 27 - protein, 276 aa, Artificial Sequence
  E6_VH7 Vk9 complete with IGk secretory signal and c-myc peptide
MGDNDIHFAFLSTGVHSQVQLQQSGGGLVQPGGSMKLSCVASGFTSSNYWLNWVRQSPERGLEWVAEIRLKSNNYATNYAESVKGRFTISRDDSKSSVYLQVNNLRAEDTGIYYCTRSTARATPYYFDYWGQGTTVTVSSGGGGSGGGGSGGGGSDIELTQSPSSLAVSAGEKVTMSCKSSQSLLNSRARKNFLTWYQQKPGQSPKLLIYWASTRESGVPDRFTGSGSGTDFTLTISSVQAEDLAVYYCKQSYNLYTFGGGTKLEEQKLISEEDLN

SEQ ID NO: 28 - protein, 245 aa, Artificial Sequence
  E6_VH7 Vk9 full
LQQSGGGLVQPGGSMKLSCVASGFTSSNYWLNWVRQSPERGLEWVAEIRLKSNNYATNYAESVKGRFTISRDDSKSSVYLQVNNLRAEDTGIYYCTRSTARATPYYFDYWGQGTTVTVSSGGGGSGGGGSGGGGSDIELTQSPSSLAVSAGEKVTMSCKSSQSLLNSRARKNFLTWYQQKPGQSPKLLIYWASTRESGVPDRFTGSGSGTDFTLTISSVQAEDLAVYYCKQSYNLYTFGGGTKLE

SEQ ID NO: 29 - protein, 250 aa, Artificial Sequence
  C10_VH3 Vk3 complete with IGk secretory signal and c-myc peptide
MGDNDIHFAFLSTGVHSQVQLQESGGGLVQPGGSRKLSCAASGFTFSSFGMHWVRQAPEKGLEWVAYISSGSSTLHYADTVKGRFTISRDNPKNTLFLQMKLPSLCYGLLGPRDHGHSSGGGGSGGGGSGGGGSELTQSPASLAVSLGQRATISYRASKSVSTSGYSYMHWNQQKPGQPPRLLIYLVSNLESGVPARFSGSGSGTDFTLNIHPVEEEDAATYYCQHIRELTRSEGAPSSEQKLISEEDLN

SEQ ID NO: 30 - protein, 219 aa, Artificial Sequence
  C10_VH3 Vk3 full
LQESGGGLVQPGGSRKLSCAASGFTFSSFGMHWVRQAPEKGLEWVAYISSGSSTLHYADTVKGRFTISRDNPKNTLFLQMKLPSLCYGLLGPRDHGHSSGGGGSGGGGSGGGGSELTQSPASLAVSLGQRATISYRASKSVSTSGYSYMHWNQQKPGQPPRLLIYLVSNLESGVPARFSGSGSGTDFTLNIHPVEEEDAATYYCQHIRELTRSEGAPSS

SEQ ID NO: 31 - protein, 250 aa, Artificial Sequence
  C10_VH4 Vk3 complete with IGk secretory signal and c-myc peptide
MGDNDIHFAFLSTGVHSQVQLQQSGGGLVQPGGSRKLSCAASGFTFSSFGMHWVRQAPEKGLEWVAYISSGSSTLHYADTVKGRFTISRDNPKNTLFLQMKLPSLCYGLLGPRDHGHSSGGGGSGGGGSGGGGSELTQSPASLAVSLGQRATISYRASKSVSTSGYSYMHWNQQKPGQPPRLLIYLVSNLESGVPARFSGSGSGTDFTLNIHPVEEEDAATYYCQHIRELTRSEGAPSSEQKLISEEDLN

SEQ ID NO: 32 - protein, 219 aa, Artificial Sequence
  C10_VH4 Vk3 full
LQQSGGGLVQPGGSRKLSCAASGFTFSSFGMHWVRQAPEKGLEWVAYISSGSSTLHYADTVKGRFTISRDNPKNTLFLQMKLPSLCYGLLGPRDHGHSSGGGGSGGGGSGGGGSELTQSPASLAVSLGQRATISYRASKSVSTSGYSYMHWNQQKPGQPPRLLIYLVSNLESGVPARFSGSGSGTDFTLNIHPVEEEDAATYYCQHIRELTRSEGAPSS

SEQ ID NO: 33 - DNA, 354 bp, Artificial Sequence
  E6_VH1 heavy chain variable region
ctgcaggagtctggaggaggcttggtgcaacctggaggatccatgaaactctcctgtgttgcctctggattcacttccagtaactactggttgaactgggtccgccagtctccagagagggggcttgagtgggttgctgaaattagattgaaatctaataattatgcaacaaattatgcggagtctgtgaaagggaggttcaccatctcaagagacgattccaaaagtagtgtctacctgcaagtgaacaacttaagagctgaagacactggcatttattactgtaccaggtcaacagctcgggctaccccatactactttgactactggggccaagggaccacggtcaccgtc

SEQ ID NO: 34 - DNA, 353 bp, Artificial Sequence
  E6_VH7 heavy chain variable region
ctgcagcagtctggaggaggcttggtgcaacctggaggatccatgaaactctcctgtgttgcctctggattcacttccagtaactactggttgaactgggtccgccagtctccagagagggggcttgagtgggttgctgaaattagattgaaatctaataattatgcaacaaattatgcggagtctgtgaaagggaggttcaccatctcaagagacgattccaaaagtagtgtctacctgcaagtgaacaacttaagagctgaagacactggcatttattactgtaccaggtcaacagctcgggctaccccatactactttgactactggggccaagggaccacggtcacctc

SEQ ID NO: 35 - DNA, 324 bp, Artificial Sequence
  E6_Vk9 light chain variable region
gagctcacccagtctccatcctccctggctgtgtcagccggagagaaggtcactatgagctgcaaatccagtcagagtctgctcaacagtagagcccgaaagaacttcttgacttggtaccagcagaaaccagggcagtctcctaaattgctgatctattgggcatccactagggaatctggggtccctgatcgcttcacaggcagtggatctgggacagatttcactctcaccatcagcagtgtgcaggctgaagacctggcagtttattactgcaaacagtcttataatctgtacacgttcggagggggcaccaagctcgag

SEQ ID NO: 36 - DNA, 292 bp, Artificial Sequence
  C10_VH3 heavy chain variable region
ctgcaggagtctgggggaggcttagtgcagcctggagggtcccggaaactctcctgtgcagcctctggattcactttcagtagctttggaatgcactgggttcgtcaggctccagagaaggggctggagtgggtcgcatacattagtagtggcagtagtaccctccactatgcagacacagtgaagggccgattcaccatctccagagacaatcccaagaacaccctgttcctgcaaatgaaactaccctcactatgctatggactactggggccaagggaccacggtcacc

SEQ ID NO: 37 - DNA, 292 bp, Artificial Sequence
  C10_VH4 heavy chain variable region
ctgcagcagtcagggggaggcttagtgcagcctggagggtcccggaaactctcctgtgcagcctctggattcactttcagtagctttggaatgcactgggttcgtcaggctccagagaaggggctggagtgggtcgcatacattagtagtggcagtagtaccctccactatgcagacacagtgaagggccgattcaccatctccagagacaatcccaagaacaccctgttcctgcaaatgaaactaccctcactatgctatggactactggggccaagggaccacggtcacc

SEQ ID NO: 38 - DNA, 317 bp, Artificial Sequence
  C10_Vk3 light chain variable region
gagctcacccagtctcctgcttccttagctgtatctctggggcagagggccaccatctcatacagggccagcaaaagtgtcagtacatctggctatagttatatgcactggaaccaacagaaaccaggacagccacccagactcctcatctatcttgtatccaacctagaatctggggtccctgccaggttcagtggcagtgggtctgggacagacttcaccctcaacatccatcctgtggaggaggaggatgctgcaacctattactgtcagcacattagggagcttacacgttcggagggggcaccaagctcgag

SEQ ID NO: 39 - DNA, 836 bp, Artificial Sequence
  E6_VH1 Vk9 clone complete with Igk secretion signal and c-myc peptide
atgggtgacaatgacatccactttgcctttctctccacaggtgtccactcccaggtccactgcaggagtctggaggaggcttggtgcaacctggaggatccatgaaactctcctgtgttgcctctggattcacttccagtaactactggttgaactgggtccgccagtctccagagagggggcttgagtgggttgctgaaattagattgaaatctaataattatgcaacaaattatgcggagtctgtgaaagggaggttcaccatctcaagagacgattccaaaagtagtgtctacctgcaagtgaacaacttaagagctgaagacactggcatttattactgtaccaggtcaacagctcgggctaccccatactactttgactactggggccaagggaccacggtcaccgtctcctcaggtggaggcggttcaggcggaggtggctctggcggtggcggatcggacatcgagctcacccagtctccatcctccctggctgtgtcagccggagagaaggtcactatgagctgcaaatccagtcagagtctgctcaacagtagagcccgaaagaacttcttgacttggtaccagcagaaaccagggcagtctcctaaattgctgatctattgggcatccactagggaatctggggtccctgatcgcttcacaggcagtggatctgggacagatttcactctcaccatcagcagtgtgcaggctgaagacctggcagtttattactgcaaacagtcttataatctgtacacgttcggagggggcaccaagctcgagatcaaacgggaacaaaaactcatctcagaagaggatctgaat

SEQ ID NO: 40 - DNA, 735 bp, Artificial Sequence
  E6_VH1 Vk9 clone full
ctgcaggagtctggaggaggcttggtgcaacctggaggatccatgaaactctcctgtgttgcctctggattcacttccagtaactactggttgaactgggtccgccagtctccagagagggggcttgagtgggttgctgaaattagattgaaatctaataattatgcaacaaattatgcggagtctgtgaaagggaggttcaccatctcaagagacgattccaaaagtagtgtctacctgcaagtgaacaacttaagagctgaagacactggcatttattactgtaccaggtcaacagctcgggctaccccatactactttgactactggggccaagggaccacggtcaccgtctcctcaggtggaggcggttcaggcggaggtggctctggcggtggcggatcggacatcgagctcacccagtctccatcctccctggctgtgtcagccggagagaaggtcactatgagctgcaaatccagtcagagtctgctcaacagtagagcccgaaagaacttcttgacttggtaccagcagaaaccagggcagtctcctaaattgctgatctattgggcatccactagggaatctggggtccctgatcgcttcacaggcagtggatctgggacagatttcactctcaccatcagcagtgtgcaggctgaagacctggcagtttattactgcaaacagtcttataatctgtacacgttcggagggggcaccaagctcgag

SEQ ID NO: 41 - DNA, 835 bp, Artificial Sequence
  E6_VH7 Vk9 clone complete with Igk secretion signal and c-myc peptide
atgggtgacaatgacatccactttgcctttctctccacaggtgtccactcccaggtccactgcagcagtctggaggaggcttggtgcaacctggaggatccatgaaactctcctgtgttgcctctggattcacttccagtaactactggttgaactgggtccgccagtctccagagagggggcttgagtgggttgctgaaattagattgaaatctaataattatgcaacaaattatgcggagtctgtgaaagggaggttcaccatctcaagagacgattccaaaagtagtgtctacctgcaagtgaacaacttaagagctgaagacactggcatttattactgtaccaggtcaacagctcgggctaccccatactactttgactactggggccaagggaccacggtcacctctcctcaggtggaggcggttcaggcggaggtggctctggcggtggcggatcggacatcgagctcacccagtctccatcctccctggctgtgtcagccggagagaaggtcactatgagctgcaaatccagtcagagtctgctcaacagtagagcccgaaagaacttcttgacttggtaccagcagaaaccagggcagtctcctaaattgctgatctattgggcatccactagggaatctggggtccctgatcgcttcacaggcagtggatctgggacagatttcactctcaccatcagcagtgtgcaggctgaagacctggcagtttattactgcaaacagtcttataatctgtacacgttcggagggggcaccaagctcgagatcaaacgggaacaaaaactcatctcagaagaggatctgaat

SEQ ID NO: 42 - DNA, 734 bp, Artificial Sequence
  E6_VH7 Vk9 clone full
ctgcagcagtctggaggaggcttggtgcaacctggaggatccatgaaactctcctgtgttgcctctggattcacttccagtaactactggttgaactgggtccgccagtctccagagagggggcttgagtgggttgctgaaattagattgaaatctaataattatgcaacaaattatgcggagtctgtgaaagggaggttcaccatctcaagagacgattccaaaagtagtgtctacctgcaagtgaacaacttaagagctgaagacactggcatttattactgtaccaggtcaacagctcgggctaccccatactactttgactactggggccaagggaccacggtcacctctcctcaggtggaggcggttcaggcggaggtggctctggcggtggcggatcggacatcgagctcacccagtctccatcctccctggctgtgtcagccggagagaaggtcactatgagctgcaaatccagtcagagtctgctcaacagtagagcccgaaagaacttcttgacttggtaccagcagaaaccagggcagtctcctaaattgctgatctattgggcatccactagggaatctggggtccctgatcgcttcacaggcagtggatctgggacagatttcactctcaccatcagcagtgtgcaggctgaagacctggcagtttattactgcaaacagtcttataatctgtacacgttcggagggggcaccaagctcgag

SEQ ID NO: 43 - DNA, 767 bp, Artificial Sequence
  C10_VH3 Vk3 clone complete with Igk secretion signal and c-myc peptide
atgggtgacaatgacatccactttgcctttctctccacaggtgtccactcccaggtccactgcaggagtctgggggaggcttagtgcagcctggagggtcccggaaactctcctgtgcagcctctggattcactttcagtagctttggaatgcactgggttcgtcaggctccagagaaggggctggagtgggtcgcatacattagtagtggcagtagtaccctccactatgcagacacagtgaagggccgattcaccatctccagagacaatcccaagaacaccctgttcctgcaaatgaaactaccctcactatgctatggactactggggccaagggaccacggtcacctcctcaggtggaggcggttcaggcggaggtggctctggcggtggcggatcggacatcgagctcacccagtctcctgcttccttagctgtatctctggggcagagggccaccatctcatacagggccagcaaaagtgtcagtacatctggctatagttatatgcactggaaccaacagaaaccaggacagccacccagactcctcatctatcttgtatccaacctagaatctggggtccctgccaggttcagtggcagtgggtctgggacagacttcaccctcaacatccatcctgtggaggaggaggatgctgcaacctattactgtcagcacattagggagcttacacgttcggagggggcaccaagctcgagatcaaacgggaacaaaaactcatctcagaagaggatctgaat

SEQ ID NO: 44 - DNA, 666 bp, Artificial Sequence
  C10_VH3 Vk3 full clone
ctgcaggagtctgggggaggcttagtgcagcctggagggtcccggaaactctcctgtgcagcctctggattcactttcagtagctttggaatgcactgggttcgtcaggctccagagaaggggctggagtgggtcgcatacattagtagtggcagtagtaccctccactatgcagacacagtgaagggccgattcaccatctccagagacaatcccaagaacaccctgttcctgcaaatgaaactaccctcactatgctatggactactggggccaagggaccacggtcacctcctcaggtggaggcggttcaggcggaggtggctctggcggtggcggatcggacatcgagctcacccagtctcctgcttccttagctgtatctctggggcagagggccaccatctcatacagggccagcaaaagtgtcagtacatctggctatagttatatgcactggaaccaacagaaaccaggacagccacccagactcctcatctatcttgtatccaacctagaatctggggtccctgccaggttcagtggcagtgggtctgggacagacttcaccctcaacatccatcctgtggaggaggaggatgctgcaacctattactgtcagcacattagggagcttacacgttcggagggggcaccaagctcgag

SEQ ID NO: 45 - DNA, 767 bp, Artificial Sequence
  C10_VH4 Vk3 clone complete with Igk secretion signal and c-myc peptide
atgggtgacaatgacatccactttgcctttctctccacaggtgtccactcccaggtccactgcagcagtcagggggaggcttagtgcagcctggagggtcccggaaactctcctgtgcagcctctggattcactttcagtagctttggaatgcactgggttcgtcaggctccagagaaggggctggagtgggtcgcatacattagtagtggcagtagtaccctccactatgcagacacagtgaagggccgattcaccatctccagagacaatcccaagaacaccctgttcctgcaaatgaaactaccctcactatgctatggactactggggccaagggaccacggtcacctcctcaggtggaggcggttcaggcggaggtggctctggcggtggcggatcggacatcgagctcacccagtctcctgcttccttagctgtatctctggggcagagggccaccatctcatacagggccagcaaaagtgtcagtacatctggctatagttatatgcactggaaccaacagaaaccaggacagccacccagactcctcatctatcttgtatccaacctagaatctggggtccctgccaggttcagtggcagtgggtctgggacagacttcaccctcaacatccatcctgtggaggaggaggatgctgcaacctattactgtcagcacattagggagcttacacgttcggagggggcaccaagctcgagatcaaacgggaacaaaaactcatctcagaagaggatctgaat

SEQ ID NO: 46 - DNA, 666 bp, Artificial Sequence
  C10_VH4 Vk3 clone full
ctgcagcagtcagggggaggcttagtgcagcctggagggtcccggaaactctcctgtgcagcctctggattcactttcagtagctttggaatgcactgggttcgtcaggctccagagaaggggctggagtgggtcgcatacattagtagtggcagtagtaccctccactatgcagacacagtgaagggccgattcaccatctccagagacaatcccaagaacaccctgttcctgcaaatgaaactaccctcactatgctatggactactggggccaagggaccacggtcacctcctcaggtggaggcggttcaggcggaggtggctctggcggtggcggatcggacatcgagctcacccagtctcctgcttccttagctgtatctctggggcagagggccaccatctcatacagggccagcaaaagtgtcagtacatctggctatagttatatgcactggaaccaacagaaaccaggacagccacccagactcctcatctatcttgtatccaacctagaatctggggtccctgccaggttcagtggcagtgggtctgggacagacttcaccctcaacatccatcctgtggaggaggaggatgctgcaacctattactgtcagcacattagggagcttacacgttcggagggggcaccaagctcgag

SEQ ID NO: 47 - protein, 17 aa, Artificial Sequence
  Linker signal
SSGGGGSGGGGSGGGGS

SEQ ID NO: 48 - protein, 20 aa, Artificial Sequence
  Secretory signal
MGDNDIHFAFLSTGVHSQVQ

SEQ ID NO: 49 - protein, 414 aa, Human
MSEYIRVTEDENDEPIEIPSEDDGTVLLSTVTAQFPGACGLRYRNPVSQCMRGVRLVEGILHAPDAGWGNLVYVVNYPKDNKRKMDETDASSAVKVKRAVQKTSDLIVLGLPWKTTEQDLKEYFSTFGEVLMVQVKKDLKTGHSKGFGFVRFTEYETQVKVMSQRHMIDGRWCDCKLPNSKQSQDEPLRSRKVFVGRCTEDMTEDELREFFSQYGDVMDVFIPKPFRAFAFVTFADDQIAQSLCGEDLIIKGISVHISNAEPKHNSNRQLERSGRFGGNPGGFGNQGGFGNSRGGGAGLGNNQGSNMGGGMNFGAFSINPAMMAAAQAALQSSWGMMGMLASQQNQSGPSGNNQNQGNMQREPNQAFGSGNNSYSGSNSGAAIGWGSASNAGSGSGFNGGFGSSMDSKSSGWGM

SEQ ID NO: 50 - protein, 551 aa, Human
MDELFPLIFPAEPAQASGPYVEIIEQPKQRGMRFRYKCEGRSAGSIPGERSTDTTKTHPTIKINGYTGPGTVRISLVTKDPPHRPHPHELVGKDCRDGFYEAELCPDRCIHSFQNLGIQCVKKRDLEQAISQRIQTNNNPFQVPIEEQRGDYDLNAVRLCFQVTVRDPSGRPLRLPPVLPHPIFDNRAPNTAELKICRVNRNSGSCLGGDEIFLLCDKVQKEDIEVYFTGPGWEARGSFSQADVHRQVAIVFRTPPYADPSLQAPVRVSMQLRRPSDRELSEPMEFQYLPDTDDRHRIEEKRKRTYETFKSIMKKSPFSGPTDPRPPPRRIAVPSRSSASVPKPAPQPYPFTSSLSTINYDEFPTMVFPSGQISQASALAPAPPQVLPQAPAPAPAPAMVSALAQAPAPVPVLAPGPPQAVAPPAPKPTQAGEGTLSEALLQLQFDDEDLGALLGNSTDPAVFTDLASVDNSEFQQLLNQGIPVAPHTTEPMLMEYPEAITRLVTGAQRPPDPAPAPLGAPGLPNGLLSGDEDFSSIADMDFSALLSQISS

SEQ ID NO: 51 - protein, 17 aa, Artificial Sequence
  stanniocalcin signal sequence
MLQNSAVLLLLVISASA

SEQ ID NO: 52 - protein, 22 aa, Artificial Sequence
  signal sequence
MPTWAWWLFLVLLLALWAPARG

SEQ ID NO: 53 - protein, 20 aa, Artificial Sequence
  Ig  secretory signal
MGDNDIHFAFLSTGVHSQVQ